European Patent Specification EP 3 844 503 B1, published May 29, 2024. Title: TK-1 in prognostic indices for DLBCL. Applicant: Roche Diagnostics  Operations Inc. The sequence listing filed with the application follows.

SEQUENCE LISTING (10 sequences)

SEQ ID NO: 1 - protein, 234 aa, Homo sapiens
MSCINLPTVLPGSPSKTRGQIQVILGPMFSGKSTELMRRVRRFQIAQYKCLVIKYAKDTRYSSSFCTHDRNTMEALPACLLRDVAQEALGVAVIGIDEGQFFPDIVEFCEAMANAGKTVIVAALDGTFQRKPFGAILNLVPLAESVVKLTAVCMECFREAAYTKRLGTEKEVEVIGGADKYHSVCRLCYFKKASGQPAGPDNKENCPVPGKPGEAVAARKLFAPQQILQCSPAN

SEQ ID NO: 2 - protein, 31 aa, Homo sapiens
GQPAGPDNKENCPVPGKPGEAVAARKLFAPQ

SEQ ID NO: 3 - protein, 185 aa, Artificial Sequence
  synthesized based rabbit MAB 6C6 heavy chain
METGLRWLLLVAVLKGVQCQEQLEESGGDLVKPEGSLTLTCTASRFSFSSSYWICWVRQAPGKGLEWIACIYAGDSGSSYYASWAKGRFTVSKTSSTTVTLQTTSLTAADTATYFCARASVGAAYDYFALWGPGTLVTVSSGQPKAPSVFPLAPCCGDTPSSTVTLGCLVKGYLPEPVTVTWNSG

SEQ ID NO: 4 - protein, 236 aa, Artificial Sequence
  synthesized based on rabbit MAB 6C6 light chain
MDTRAPTQLLGLLLLWLPGARCALVMTQTPASVEAAMGGTVTIKCQASEDVSSHLAWYQQRPGQPPKLLIYGASDLASGVPSRFTGSGSGTQFTLAISDLECADAATYYCQGYYYISDSPYVFGGGTEVVVKGDPVAPTVLIFPPAADQVATGTVTIVCVANKYFPDVTVTWEVDGTTQTTGIENSKTPQNSADCTYNLSSTLTLTSTQYNSHKEYTCKVTQGTTSVVQSFNRGDC

SEQ ID NO: 5 - protein, 265 aa, Homo sapiens
MLLWPLRGWAARALRCFGPGSRGSPASGPGPRRVQRRAWPPDKEQEKEKKSVICVEGNIASGKTTCLEFFSNATDVEVLTEPVSKWRNVRGHNPLGLMYHDASRWGLTLQTYVQLTMLDRHTRPQVSSVRLMERSIHSARYIFVENLYRSGKMPEVDYVVLSEWFDWILRNMDVSVDLIVYLRTNPETCYQRLKKRCREEEKVIPLEYLEAIHHLHEEWLIKGSLFPMAAPVLVIEADHHMERMLELFEQNRDRILTPENRKHCP

SEQ ID NO: 6 - protein, 20 aa, Homo sapiens
KPGEAVAARKLFAPQQILQC

SEQ ID NO: 7 - protein, 187 aa, Artificial Sequence
  synthesized based on rabbit MAB 4H4 heavy chain
METGLRWLLLVAVLKGVQCQSLEESGGGLVQPEGSLTLTCTASGFSFSSGYDMCWVRQTPGKGLEWIACISVDSDGVTYYASWAKGRFTISKTSSTTVTLQMTSLTAADTATYFCARGYESSSGVYIPYFTLWGPGTLVTVSSGQPKAPSVFPLAPCCGDTPSSTVTLGCLVKGYLPEPVTVTWNSG

SEQ ID NO: 8 - protein, 238 aa, Artificial Sequence
  synthesized based on rabbit MAB 4H4 light chain
MDMRAPTQLLGLLLLWLPGARCADIVLTQTPASVEAAVGGTVTIKCQASQSIYSYLAWYQHKPGQPPKLLIYKASTLASGVPSRFKGSGSGTEYTLTISDLECADAATYYCQHYYYSSTSGGGVFGGGTEVVVKGDPVAPTVLIFPPAADQVATGTVTIVCVANKYFPDVTVTWEVDGTTQTTGIENSKTPQNSADCTYNLSSTLTLTSTQYNSHKEYTCKVTQGTTSVVQSFNRGDC

SEQ ID NO: 9 - protein, 179 aa, Artificial Sequence
  synthesized based on rabbit MAB 23C11 heavy chain
METGLRWLLLVAVLKGVQCQSLEESGGRLVTPGTPLTLTCTASGFSLSNYYMSWVRQAPGKGLEWIGIIYGDDNTYCANWTKGRFTISKTSTTVDLTITSPTTEDTATYFCARGPDYIAAKMDIWGPGTLVTVSLGQPKAPSVFPLAPCCGDTPSSTVTLGCLVKGYLPEPVTVTWNSG

SEQ ID NO: 10 - protein, 239 aa, Artificial Sequence
  synthesized based on rabbit MAB 23C11 light chain
MDTRAPTQLLGLLLLWLPGARCDVVMTQTPASVEAAVGGTVTIKCQASQSISGYLSWYQQKPGQRPKLLIYRASTLESGVPSRFKGSGSGTEFTLTISDLECADAATYYCQCTYGSSTFSSYGNAFGGGTEVVVKGDPVAPTVLIFPPAADQVATGTVTIVCVANKYFPDVTVTWEVDGTTQTTGIENSKTPQNSADCTYNLSSTLTLTSTQYNSHKEYTCKVTQGTTSVVQSFNRGDC